European Patent Specification EP 3 423 452 B1, published May 7, 2025. Title: WNT Signaling Pathway Inhibitors for Treatments of Disease. Applicant: University of Maryland, Baltimore XUE, Fengtian SHU, Yan. The sequence listing filed with the application follows.

SEQUENCE LISTING (6 sequences)

SEQ ID NO: 1 - DNA, 18 bp, Artificial Sequence
  Synthetic sequence (primer)
ctccttggaggcaagagc

SEQ ID NO: 2 - DNA, 18 bp, Artificial Sequence
  Synthetic sequence (primer)
ggccacgcagcaccgctg

SEQ ID NO: 3 - DNA, 21 bp, Artificial Sequence
  Synthetic sequence (primer)
aaggcggaggagacctgcgcg

SEQ ID NO: 4 - DNA, 18 bp, Artificial Sequence
  Synthetic sequence (primer)
atcgtgcggcattgcggc

SEQ ID NO: 5 - DNA, 20 bp, Artificial Sequence
  Synthetic sequence (primer)
accacagtccatgccatcac

SEQ ID NO: 6 - DNA, 19 bp, Artificial Sequence
  Synthetic sequence (primer)
tccaccaccctgttgctgt